European Patent Application EP 4 123 026 A1, published January 25, 2023. Title: Nucleic acid construct and agent for treatment or diagnosis of mismatch repair-deficient cancers comprising the same. Applicant: Public University Corporation Yokohama City University. The sequence listing filed with the application follows.

SEQUENCE LISTING (83 sequences)

SEQ ID NO: 1 - DNA, 45 bp, Artificial Sequence
  primer DTA-Fw
actcactataggctagcgtcctcgccatggatcctgatgatgttg

SEQ ID NO: 2 - DNA, 60 bp, Artificial Sequence
  primer SSA-5'DTA-Rv
ccgccccgactctagaatgcattaccctgttatccctatcattgtgtaccagattttggc

SEQ ID NO: 3 - DNA, 48 bp, Artificial Sequence
  primer SSA-3'DTA-Fw
tagggataacagggtaatgcatcttttgtgatggaaaacttttcttcg

SEQ ID NO: 4 - DNA, 46 bp, Artificial Sequence
  primer DTA-Rv
ccgccccgactctagaatcacaaagatcgcctgacacgatttcctg

SEQ ID NO: 5 - DNA, 23 bp, Artificial Sequence
  primer Nluc-Fw
taatacgactcactataggctag

SEQ ID NO: 6 - DNA, 44 bp, Artificial Sequence
  primer SSA-5'Nluc-Rv
ggccgccccgactctagaatcacggccgtccgaaatagtcgatc

SEQ ID NO: 7 - DNA, 41 bp, Artificial Sequence
  primer SSA-3'Nluc-Fw
cggccgtgattctagatgcataccctgtggatgatcatcac

SEQ ID NO: 8 - DNA, 23 bp, Artificial Sequence
  primer Nluc-Rv
ccgccccgactctagagtcgcgg

SEQ ID NO: 9 - DNA, 591 bp, Corynebacterium diphtheriae
  CDS (1)..(591)
atggatcctgatgatgttgttgattcttctaaatcttttgtgatggaaaacttttcttcgtaccacgggactaaacctggttatgtagattccattcaaaaaggtatacaaaagccaaaatctggtacacaaggaaattatgacgatgattggaaagggttttatagtaccgacaataaatacgacgctgcgggatactctgtagataatgaaaacccgctctctggaaaagctggaggcgtggtcaaagtgacgtatccaggactgacgaaggttctcgcactaaaagtggataatgccgaaactattaagaaagagttaggtttaagtctcactgaaccgttgatggagcaagtcggaacggaagagtttatcaaaaggttcggtgatggtgcttcgcgtgtagtgctcagccttcccttcgctgaggggagttctagcgttgaatatattaataactgggaacaggcgaaagcgttaagcgtagaacttgagattaattttgaaacccgtggaaaacgtggccaagatgcgatgtatgagtatatggctcaagcctgtgcaggaaatcgtgtcaggcgatctttgtga

SEQ ID NO: 10 - protein, 196 aa, Corynebacterium diphtheriae
MDPDDVVDSSKSFVMENFSSYHGTKPGYVDSIQKGIQKPKSGTQGNYDDDWKGFYSTDNKYDAAGYSVDNENPLSGKAGGVVKVTYPGLTKVLALKVDNAETIKKELGLSLTEPLMEQVGTEEFIKRFGDGASRVVLSLPFAEGSSSVEYINNWEQAKALSVELEINFETRGKRGQDAMYEYMAQACAGNRVRRSL

SEQ ID NO: 11 - DNA, 132 bp, Artificial Sequence
  5'DT-A fragment
  CDS (1)..(132)
atggatcctgatgatgttgttgattcttctaaatcttttgtgatggaaaacttttcttcgtaccacgggactaaacctggttatgtagattccattcaaaaaggtatacaaaagccaaaatctggtacacaa

SEQ ID NO: 12 - protein, 44 aa, Artificial Sequence
  Synthetic Construct
MDPDDVVDSSKSFVMENFSSYHGTKPGYVDSIQKGIQKPKSGTQ

SEQ ID NO: 13 - DNA, 556 bp, Artificial Sequence
  3'DT-A fragment
  CDS (2)..(556)
atcttttgtgatggaaaacttttcttcgtaccacgggactaaacctggttatgtagattccattcaaaaaggtatacaaaagccaaaatctggtacacaaggaaattatgacgatgattggaaagggttttatagtaccgacaataaatacgacgctgcgggatactctgtagataatgaaaacccgctctctggaaaagctggaggcgtggtcaaagtgacgtatccaggactgacgaaggttctcgcactaaaagtggataatgccgaaactattaagaaagagttaggtttaagtctcactgaaccgttgatggagcaagtcggaacggaagagtttatcaaaaggttcggtgatggtgcttcgcgtgtagtgctcagccttcccttcgctgaggggagttctagcgttgaatatattaataactgggaacaggcgaaagcgttaagcgtagaacttgagattaattttgaaacccgtggaaaacgtggccaagatgcgatgtatgagtatatggctcaagcctgtgcaggaaatcgtgtcaggcgatctttg

SEQ ID NO: 14 - protein, 185 aa, Artificial Sequence
  Synthetic Construct
SFVMENFSSYHGTKPGYVDSIQKGIQKPKSGTQGNYDDDWKGFYSTDNKYDAAGYSVDNENPLSGKAGGVVKVTYPGLTKVLALKVDNAETIKKELGLSLTEPLMEQVGTEEFIKRFGDGASRVVLSLPFAEGSSSVEYINNWEQAKALSVELEINFETRGKRGQDAMYEYMAQACAGNRVRRSL

SEQ ID NO: 15 - DNA, 23 bp, Artificial Sequence
  23 bp sequence inserted between 5'DT-A and 3'DT-A fragments
tgatagggataacagggtaatgc

SEQ ID NO: 16 - DNA, 714 bp, Artificial Sequence
  sequence of [5'DT-A fragment] + [3'DT-A fragment] in the SA-DTA construct
atggatcctgatgatgttgttgattcttctaaatcttttgtgatggaaaacttttcttcgtaccacgggactaaacctggttatgtagattccattcaaaaaggtatacaaaagccaaaatctggtacacaatgatagggataacagggtaatgcatcttttgtgatggaaaacttttcttcgtaccacgggactaaacctggttatgtagattccattcaaaaaggtatacaaaagccaaaatctggtacacaaggaaattatgacgatgattggaaagggttttatagtaccgacaataaatacgacgctgcgggatactctgtagataatgaaaacccgctctctggaaaagctggaggcgtggtcaaagtgacgtatccaggactgacgaaggttctcgcactaaaagtggataatgccgaaactattaagaaagagttaggtttaagtctcactgaaccgttgatggagcaagtcggaacggaagagtttatcaaaaggttcggtgatggtgcttcgcgtgtagtgctcagccttcccttcgctgaggggagttctagcgttgaatatattaataactgggaacaggcgaaagcgttaagcgtagaacttgagattaattttgaaacccgtggaaaacgtggccaagatgcgatgtatgagtatatggctcaagcctgtgcaggaaatcgtgtcaggcgatctttgtga

SEQ ID NO: 17 - DNA, 556 bp, Artificial Sequence
  3'DT-A fragment, 95% homology
atcttttgtgatggaaaatttttcttcgtaccacggcactaaacctggttacgtagattccattcagaaaggtatacaaaaaccaaaatctggtacacaaggaaattatgacgatgattggaaagggttttatagtaccgacaataaatacgacgctgcgggatactctgtagataatgaaaacccgctctctggaaaagctggaggcgtggtcaaagtgacgtatccaggactgacgaaggttctcgcactaaaagtggataatgccgaaactattaagaaagagttaggtttaagtctcactgaaccgttgatggagcaagtcggaacggaagagtttatcaaaaggttcggtgatggtgcttcgcgtgtagtgctcagccttcccttcgctgaggggagttctagcgttgaatatattaataactgggaacaggcgaaagcgttaagcgtagaacttgagattaattttgaaacccgtggaaaacgtggccaagatgcgatgtatgagtatatggctcaagcctgtgcaggaaatcgtgtcaggcgatctttg

SEQ ID NO: 18 - DNA, 556 bp, Artificial Sequence
  3'DT-A fragment, 90% homology
atcttttgtcatggaaaatttttcttcctaccacggcactaaaccaggttatgttgattccatccaaaaaggaatacaaaaaccaaaatcaggtacacaaggaaattatgacgatgattggaaagggttttatagtaccgacaataaatacgacgctgcgggatactctgtagataatgaaaacccgctctctggaaaagctggaggcgtggtcaaagtgacgtatccaggactgacgaaggttctcgcactaaaagtggataatgccgaaactattaagaaagagttaggtttaagtctcactgaaccgttgatggagcaagtcggaacggaagagtttatcaaaaggttcggtgatggtgcttcgcgtgtagtgctcagccttcccttcgctgaggggagttctagcgttgaatatattaataactgggaacaggcgaaagcgttaagcgtagaacttgagattaattttgaaacccgtggaaaacgtggccaagatgcgatgtatgagtatatggctcaagcctgtgcaggaaatcgtgtcaggcgatctttg

SEQ ID NO: 19 - DNA, 556 bp, Artificial Sequence
  3'DT-A fragment, 80% homology
atctttcgtcatggagaatttttcatcctaccatggcactaagccaggttacgttgattctatccaaaagggaatacagaaaccaaagtcaggtacacaaggaaattatgacgatgattggaaagggttttatagtaccgacaataaatacgacgctgcgggatactctgtagataatgaaaacccgctctctggaaaagctggaggcgtggtcaaagtgacgtatccaggactgacgaaggttctcgcactaaaagtggataatgccgaaactattaagaaagagttaggtttaagtctcactgaaccgttgatggagcaagtcggaacggaagagtttatcaaaaggttcggtgatggtgcttcgcgtgtagtgctcagccttcccttcgctgaggggagttctagcgttgaatatattaataactgggaacaggcgaaagcgttaagcgtagaacttgagattaattttgaaacccgtggaaaacgtggccaagatgcgatgtatgagtatatggctcaagcctgtgcaggaaatcgtgtcaggcgatctttg

SEQ ID NO: 20 - DNA, 556 bp, Artificial Sequence
  3'DT-A fragment, 70% homology
atcattcgtcatggagaatttctcatcctatcatggcaccaagccaggatacgttgactctatccagaagggaattcagaaacctaagtcaggcacacaaggaaattatgacgatgattggaaagggttttatagtaccgacaataaatacgacgctgcgggatactctgtagataatgaaaacccgctctctggaaaagctggaggcgtggtcaaagtgacgtatccaggactgacgaaggttctcgcactaaaagtggataatgccgaaactattaagaaagagttaggtttaagtctcactgaaccgttgatggagcaagtcggaacggaagagtttatcaaaaggttcggtgatggtgcttcgcgtgtagtgctcagccttcccttcgctgaggggagttctagcgttgaatatattaataactgggaacaggcgaaagcgttaagcgtagaacttgagattaattttgaaacccgtggaaaacgtggccaagatgcgatgtatgagtatatggctcaagcctgtgcaggaaatcgtgtcaggcgatctttg

SEQ ID NO: 21 - DNA, 513 bp, Artificial Sequence
  NanoLuc (Nluc) gene encoding modified luciferase
  CDS (1)..(513)
atggtcttcacactcgaagatttcgttggggactggcgacagacagccggctacaacctggaccaagtccttgaacagggaggtgtgtccagtttgtttcagaatctcggggtgtccgtaactccgatccaaaggattgtcctgagcggtgaaaatgggctgaagatcgacatccatgtcatcatcccgtatgaaggtctgagcggcgaccaaatgggccagatcgaaaaaatttttaaggtggtgtaccctgtggatgatcatcactttaaggtgatcctgcactatggcacactggtaatcgacggggttacgccgaacatgatcgactatttcggacggccgtatgaaggcatcgccgtgttcgacggcaaaaagatcactgtaacagggaccctgtggaacggcaacaaaattatcgacgagcgcctgatcaaccccgacggctccctgctgttccgagtaaccatcaacggagtgaccggctggcggctgtgcgaacgcattctggcg

SEQ ID NO: 22 - protein, 171 aa, Artificial Sequence
  Synthetic Construct
MVFTLEDFVGDWRQTAGYNLDQVLEQGGVSSLFQNLGVSVTPIQRIVLSGENGLKIDIHVIIPYEGLSGDQMGQIEKIFKVVYPVDDHHFKVILHYGTLVIDGVTPNMIDYFGRPYEGIAVFDGKKITVTGTLWNGNKIIDERLINPDGSLLFRVTINGVTGWRLCERILA

SEQ ID NO: 23 - DNA, 345 bp, Artificial Sequence
  5'Nluc fragment
  CDS (1)..(345)
atggtcttcacactcgaagatttcgttggggactggcgacagacagccggctacaacctggaccaagtccttgaacagggaggtgtgtccagtttgtttcagaatctcggggtgtccgtaactccgatccaaaggattgtcctgagcggtgaaaatgggctgaagatcgacatccatgtcatcatcccgtatgaaggtctgagcggcgaccaaatgggccagatcgaaaaaatttttaaggtggtgtaccctgtggatgatcatcactttaaggtgatcctgcactatggcacactggtaatcgacggggttacgccgaacatgatcgactatttcggacggccg

SEQ ID NO: 24 - protein, 115 aa, Artificial Sequence
  Synthetic Construct
MVFTLEDFVGDWRQTAGYNLDQVLEQGGVSSLFQNLGVSVTPIQRIVLSGENGLKIDIHVIIPYEGLSGDQMGQIEKIFKVVYPVDDHHFKVILHYGTLVIDGVTPNMIDYFGRP

SEQ ID NO: 25 - DNA, 267 bp, Artificial Sequence
  3'Nluc fragment
  CDS (1)..(267)
taccctgtggatgatcatcactttaaggtgatcctgcactatggcacactggtaatcgacggggttacgccgaacatgatcgactatttcggacggccgtatgaaggcatcgccgtgttcgacggcaaaaagatcactgtaacagggaccctgtggaacggcaacaaaattatcgacgagcgcctgatcaaccccgacggctccctgctgttccgagtaaccatcaacggagtgaccggctggcggctgtgcgaacgcattctggcg

SEQ ID NO: 26 - protein, 89 aa, Artificial Sequence
  Synthetic Construct
YPVDDHHFKVILHYGTLVIDGVTPNMIDYFGRPYEGIAVFDGKKITVTGTLWNGNKIIDERLINPDGSLLFRVTINGVTGWRLCERILA

SEQ ID NO: 27 - DNA, 626 bp, Artificial Sequence
  sequence of [5'Nluc fragment] + [3'Nluc fragment] in the SA-Nluc construct
atggtcttcacactcgaagatttcgttggggactggcgacagacagccggctacaacctggaccaagtccttgaacagggaggtgtgtccagtttgtttcagaatctcggggtgtccgtaactccgatccaaaggattgtcctgagcggtgaaaatgggctgaagatcgacatccatgtcatcatcccgtatgaaggtctgagcggcgaccaaatgggccagatcgaaaaaatttttaaggtggtgtaccctgtggatgatcatcactttaaggtgatcctgcactatggcacactggtaatcgacggggttacgccgaacatgatcgactatttcggacggccgtgattctagatgcataccctgtggatgatcatcactttaaggtgatcctgcactatggcacactggtaatcgacggggttacgccgaacatgatcgactatttcggacggccgtatgaaggcatcgccgtgttcgacggcaaaaagatcactgtaacagggaccctgtggaacggcaacaaaattatcgacgagcgcctgatcaaccccgacggctccctgctgttccgagtaaccatcaacggagtgaccggctggcggctgtgcgaacgcattctggcg

SEQ ID NO: 28 - DNA, 267 bp, Artificial Sequence
  3'Nluc fragment, 95% homology
taccctgtggatgaccatcactttaaggtgattctgcactatggcacactcgtaatcgacggggttaccccgaacatgatcgactacttcggacggccgtatgaaggcatcgccgtgttcgacggcaaaaagatcactgtaacagggaccctgtggaacggcaacaaaattatcgacgagcgcctgatcaaccccgacggctccctgctgttccgagtaaccatcaacggagtgaccggctggcggctgtgcgaacgcattctggcg

SEQ ID NO: 29 - DNA, 267 bp, Artificial Sequence
  3'Nluc fragment, 90% homology
taccctgtggacgatcatcattttaaggtcatcctgcattatggcaccctggtaattgacggggtgacgccgaatatgatcgattatttcggccggccgtatgaaggcatcgccgtgttcgacggcaaaaagatcactgtaacagggaccctgtggaacggcaacaaaattatcgacgagcgcctgatcaaccccgacggctccctgctgttccgagtaaccatcaacggagtgaccggctggcggctgtgcgaacgcattctggcg

SEQ ID NO: 30 - DNA, 267 bp, Artificial Sequence
  3'Nluc fragment, 78% homology
tatcctgtcgacgatcaccattttaaagtcatcctccattatggaaccctggtgattgacggcgtgacgcccaatatgattgattattttggccggccctatgaaggcatcgccgtgttcgacggcaaaaagatcactgtaacagggaccctgtggaacggcaacaaaattatcgacgagcgcctgatcaaccccgacggctccctgctgttccgagtaaccatcaacggagtgaccggctggcggctgtgcgaacgcattctggcg

SEQ ID NO: 31 - DNA, 267 bp, Artificial Sequence
  3'Nluc fragment, 68% homology
tatccagtcgacgaccaccatttcaaagtcattctccattacggaaccctcgtgattgatggcgtgacccccaatatgattgattactttggccgcccctatgaaggcatcgccgtgttcgacggcaaaaagatcactgtaacagggaccctgtggaacggcaacaaaattatcgacgagcgcctgatcaaccccgacggctccctgctgttccgagtaaccatcaacggagtgaccggctggcggctgtgcgaacgcattctggcg

SEQ ID NO: 32 - DNA, 496 bp, Artificial Sequence
  3'DT-A fragment with 40-bp homologous region, 100% homology
cattcaaaaaggtatacaaaagccaaaatctggtacacaaggaaattatgacgatgattggaaagggttttatagtaccgacaataaatacgacgctgcgggatactctgtagataatgaaaacccgctctctggaaaagctggaggcgtggtcaaagtgacgtatccaggactgacgaaggttctcgcactaaaagtggataatgccgaaactattaagaaagagttaggtttaagtctcactgaaccgttgatggagcaagtcggaacggaagagtttatcaaaaggttcggtgatggtgcttcgcgtgtagtgctcagccttcccttcgctgaggggagttctagcgttgaatatattaataactgggaacaggcgaaagcgttaagcgtagaacttgagattaattttgaaacccgtggaaaacgtggccaagatgcgatgtatgagtatatggctcaagcctgtgcaggaaatcgtgtcaggcgatctttg

SEQ ID NO: 33 - DNA, 496 bp, Artificial Sequence
  3'DT-A fragment with 40-bp homologous region, 92.5% homology
cattcaaaaaggaatacaaaaaccaaaatcaggtacacaaggaaattatgacgatgattggaaagggttttatagtaccgacaataaatacgacgctgcgggatactctgtagataatgaaaacccgctctctggaaaagctggaggcgtggtcaaagtgacgtatccaggactgacgaaggttctcgcactaaaagtggataatgccgaaactattaagaaagagttaggtttaagtctcactgaaccgttgatggagcaagtcggaacggaagagtttatcaaaaggttcggtgatggtgcttcgcgtgtagtgctcagccttcccttcgctgaggggagttctagcgttgaatatattaataactgggaacaggcgaaagcgttaagcgtagaacttgagattaattttgaaacccgtggaaaacgtggccaagatgcgatgtatgagtatatggctcaagcctgtgcaggaaatcgtgtcaggcgatctttg

SEQ ID NO: 34 - DNA, 476 bp, Artificial Sequence
  3'DT-A fragment with 20-bp homologous region, 100% homology
agccaaaatctggtacacaaggaaattatgacgatgattggaaagggttttatagtaccgacaataaatacgacgctgcgggatactctgtagataatgaaaacccgctctctggaaaagctggaggcgtggtcaaagtgacgtatccaggactgacgaaggttctcgcactaaaagtggataatgccgaaactattaagaaagagttaggtttaagtctcactgaaccgttgatggagcaagtcggaacggaagagtttatcaaaaggttcggtgatggtgcttcgcgtgtagtgctcagccttcccttcgctgaggggagttctagcgttgaatatattaataactgggaacaggcgaaagcgttaagcgtagaacttgagattaattttgaaacccgtggaaaacgtggccaagatgcgatgtatgagtatatggctcaagcctgtgcaggaaatcgtgtcaggcgatctttg

SEQ ID NO: 35 - DNA, 476 bp, Artificial Sequence
  3'DT-A fragment with 20-bp homologous region, 95% homology
agccaaaatcaggtacacaaggaaattatgacgatgattggaaagggttttatagtaccgacaataaatacgacgctgcgggatactctgtagataatgaaaacccgctctctggaaaagctggaggcgtggtcaaagtgacgtatccaggactgacgaaggttctcgcactaaaagtggataatgccgaaactattaagaaagagttaggtttaagtctcactgaaccgttgatggagcaagtcggaacggaagagtttatcaaaaggttcggtgatggtgcttcgcgtgtagtgctcagccttcccttcgctgaggggagttctagcgttgaatatattaataactgggaacaggcgaaagcgttaagcgtagaacttgagattaattttgaaacccgtggaaaacgtggccaagatgcgatgtatgagtatatggctcaagcctgtgcaggaaatcgtgtcaggcgatctttg

SEQ ID NO: 36 - DNA, 476 bp, Artificial Sequence
  3'DT-A fragment with 20-bp homologous region, 90% homology
agccaaagtcaggtacacaaggaaattatgacgatgattggaaagggttttatagtaccgacaataaatacgacgctgcgggatactctgtagataatgaaaacccgctctctggaaaagctggaggcgtggtcaaagtgacgtatccaggactgacgaaggttctcgcactaaaagtggataatgccgaaactattaagaaagagttaggtttaagtctcactgaaccgttgatggagcaagtcggaacggaagagtttatcaaaaggttcggtgatggtgcttcgcgtgtagtgctcagccttcccttcgctgaggggagttctagcgttgaatatattaataactgggaacaggcgaaagcgttaagcgtagaacttgagattaattttgaaacccgtggaaaacgtggccaagatgcgatgtatgagtatatggctcaagcctgtgcaggaaatcgtgtcaggcgatctttg

SEQ ID NO: 37 - DNA, 476 bp, Artificial Sequence
  3'DT-A fragment with 20-bp homologous region, 85% homology
agccaaagtcaggcacacaaggaaattatgacgatgattggaaagggttttatagtaccgacaataaatacgacgctgcgggatactctgtagataatgaaaacccgctctctggaaaagctggaggcgtggtcaaagtgacgtatccaggactgacgaaggttctcgcactaaaagtggataatgccgaaactattaagaaagagttaggtttaagtctcactgaaccgttgatggagcaagtcggaacggaagagtttatcaaaaggttcggtgatggtgcttcgcgtgtagtgctcagccttcccttcgctgaggggagttctagcgttgaatatattaataactgggaacaggcgaaagcgttaagcgtagaacttgagattaattttgaaacccgtggaaaacgtggccaagatgcgatgtatgagtatatggctcaagcctgtgcaggaaatcgtgtcaggcgatctttg

SEQ ID NO: 38 - DNA, 43 bp, Artificial Sequence
  primer SSA-3'DTA-40bp-100-Fw
tagggataacagggtaatgcattcaaaaaggtatacaaaagcc

SEQ ID NO: 39 - DNA, 57 bp, Artificial Sequence
  primer SSA-3'DTA-40bp-92.5-Fw
tagggataacagggtaatgcattcaaaaaggaatacaaaaaccaaaatcaggtacac

SEQ ID NO: 40 - DNA, 45 bp, Artificial Sequence
  primer SSA-3'DTA-20bp-100-Fw
tagggataacagggtaatgcatagccaaaatctggtacacaagga

SEQ ID NO: 41 - DNA, 45 bp, Artificial Sequence
  primer SSA-3'DTA-20bp-95-Fw
tagggataacagggtaatgcatagccaaaatcaggtacacaagga

SEQ ID NO: 42 - DNA, 45 bp, Artificial Sequence
  primer SSA-3'DTA-20bp-90-Fw
tagggataacagggtaatgcatagccaaagtcaggtacacaagga

SEQ ID NO: 43 - DNA, 45 bp, Artificial Sequence
  primer SSA-3'DTA-20bp-85-Fw
tagggataacagggtaatgcatagccaaagtcaggcacacaagga

SEQ ID NO: 44 - DNA, 44 bp, Artificial Sequence
  primer Nluc-Spacer-Fw
gacggccgtgattctagaggtaccggttgacagacgttaggttg

SEQ ID NO: 45 - DNA, 40 bp, Artificial Sequence
  primer Nluc-Spacer-Rv
gatcatccacagggtatgcataaccaacagtgaaacagcg

SEQ ID NO: 46 - DNA, 45 bp, Artificial Sequence
  primer SA-5'Nluc-Rv2
caccatacgcggatcatgcatcacggccgtccgaaatagtcgatc

SEQ ID NO: 47 - DNA, 20 bp, Artificial Sequence
  primer SV40-pA-Rv
gagtgcaccatacgcggatc

SEQ ID NO: 48 - DNA, 59 bp, Artificial Sequence
  primer SA-5'DTA-Rv2
cgcggatccttatcgatgcattaccctgttatccctatcattgtgtaccagattttggc

SEQ ID NO: 49 - DNA, 23 bp, Artificial Sequence
  primer SA-3'DTA-Fw2
tgatagggataacagggtaatgc

SEQ ID NO: 50 - DNA, 20 bp, Artificial Sequence
  primer SA-TK-Fw
acacgcgtctgcgttcgacc

SEQ ID NO: 51 - DNA, 66 bp, Artificial Sequence
  primer SA-TK-Rv
atacgcgtgatgcattaccctgttatccctactcgagaatcagaggcggacttccgtggcttcttg

SEQ ID NO: 52 - DNA, 3952 bp, Artificial Sequence
  3,952 bp spacer
ggttgacagacgttaggttgtttccactgatgctccttatttctcgtacctgaaatgtccttattccctcccttcttatcccatgtttaagtcatttaagacccagctcaaacgtcacctccacaaaaccttccttgatacccctttcctcttcaattcacttggaccttttgcatttaattttaatttttattttttttaagacagagtctcactctgtcaccaggctggagtgcagtggtatgatctcagctcactaactactctgcctcccaggttcaagcaattctcatgtctcagcctcccaagtagctgggactacaggtgtgcgccaccatgcctggctaattgtgtgtgtgtgtgtgtgtatgtatgtatgtatatatgtgtgtgtgtgtatatatatatatacacaaacatatataaatatatatacatatatatatatacacacatatataaatatatatacatatatatatatacacacacacacacatatatatatatatagtttttttttttttaagtagagatggggttttgccatgttggccaggctggtctggcctcaagccatcctcccacctcggcctcgcaaagtgctggtattataggcatgagccactgtgcctggcctgcatttcattttaattataaaatattttgaactcagaaaaaagggtatgctgaatacctacgtacccacaaaagtattaacattttgccatatttgcttctgatcttattttttttgagaaattaaagatcataatacaactaaagccccatttctttcccttcattcccagaagtatgacaattatccttaaagttgatatatatcattcccatgcatgttttttatacttccctagtacaagttagctgtatcctctgctcaggggctcatcaagctgaatcaagggactcatgatcctcttcaaagttccttcaggttgttggcagaatttagttccttgtgattgtaggactgagggcccgttttctcactggctgctggccaggggttgctcccagatatttaaaggctcatgccctagcccatgacagtctcacaacatggcagctgacttcttcaaaaccagcaggagaatcttgctctagtctaccacataacctaatcacaggagcggctatcccgttattttcacagatcctggtcacattcaaggggagggaacccttctgtgtgtgtacaccaggaggcaggaattttttttttctttttcttttttgttaaaaagtcttaaagtcttttatccctaaaggaggcaggaattttgagagccatcagaattctgcctaccacagcccagaaatctgcatttttcacaagtctccagccatgatgtttctgatggctcacactgctttattccatttttaaagagtatttttattgaaaagcattagggttatggtttaaaaaatattttccctaacaaagatgggtttgtttagagtcctacttttgactaaatagctgagattcacttttatgtaaagttcattttatagcgttattaatttgggtgcctttaaaaatagtataaagcatgtttctcgagtgtagtctgttagccacctatattggagagttgggaggagagagtctctatcttgaatttatgggaaaaattctaaaatactttttataatgaaggacaacatcataactccctaataaaatgtgcatgtatatattcaaatttgctgtcattgatcctgcacctacaaaatccagtcctgggggctggcattcttactgcttgctgagggccagatgatatagattccagaatatctccatgtagattttggtgagaattactgtgctgaaaagaatgacagtattgcagttatacatgggggttttggtactttatattgtgactctgaatttaaagctatgcaatgtcttcttttttgaaaggatataattgacactggcaaaacaatgattaccctgttatccctagtcaggcagtataatccaaagatggtcaaggtcgcaaggtatgtatgacattttgacacagaatattttcctcatttgaagggggattaagtgattgcttctttttaaggataaatgttttcaactgtcattttatcttcgaaaagtaatgtaatctcatataagacttaagatataatccttttaaataattttgtcatgtgttaataaagctcataattacagtcacttccttgctaatattaacatttggttttcagcatgctaattatatcagtttgtcctgaatagcatggcagaggattttgggcccccttgcaaaattaagaataaggattccaaagcgggtgaggaagtgataggaaggggtgggccctgaagatctggacctcctggaattgagtgatgaatgctgcatcttctttgtgtctgtagtgaaattttataatgcctgcttccttttttattaagtcggcctcacctcctcaccttacctatgctgttttacttttgcttttatagttctacctgtgtttatttctcattttcgtttcatctctcaacaactctggggtggcattattattcccacttttcagataaggttactgaggcatagggaattgtccaaaggtacagagctagtccgctatagagatgagatttgaacccagggaacctggctcacagtttatgcttttgcctaccttaagtttttaatagagtgacatcaaacaaacatttaagaatatgtttttcttttccttttataatttcattaaaaacattaagtctctgatcagtctgcagtttttatgtaggggtcaggtaatgttctaacttctgctttttcctaagtgattaacaggtttttataagcccttttgaaaaaatcacggtatctgtcgagcatctttgaatcagagtaagccttctagtgagtcatatgtcagcagtttgactgtatgggcttttctaatatccagttcaagtgtttatcagtgagtttttcttttaaatagatttgggacaggtactatgagagtatataagtgatacgttataggacactaactagtatcctatgaaatggcaaaaactgcaatcacttttgcaccaaccaaatagaaactaatcagtgcacttgcttatttttctacatgctctttagggttttaaatgtcaacctactgtggcatagactttaatcctctgggtattcttttgttgttctttcctggtatatgctgtggaattgagatagactggttcgtgagcgagagattttgtgttgccacaggtaggacatgctcaaacaatacttgggtcatttcttgacccaagtcatctattcaccatagttttgtagcaccgatcttgcatacatttcatgtatcttctttgaaccccacgtcagtgctgcttatatgatactcagaaattaaacactaaggaataagattttcaggtaggattgagttttggagggtcacaaatcttgtaatgtctaatatttccactctccctgctgagaattagttttggcttccttggaggtgatatcgcctctgttgagtataagtggcctactgtgatcacaccactgcactccagcctgggtgacagagtgagaccctgtctcagaaaaaaaaaaaaaaaaaaagaatgcatggcctagatgacttctaaggtttttcccacccagttccagttttcatgttctaggcagagcagtaaagtgagaaacacatggacttgggagtttagtctcgcatttcactgccacttaatctgagcgactattccatatttaatctctctgaatgtatttactcatctttaaaggggaatgattattaacatctttttctcagggaaactatatgagtcaaggagataatatatttgaaaatctttttaactgcaaagcgctgtttcactgttggttat

SEQ ID NO: 53 - DNA, 582 bp, Artificial Sequence
  3'Nluc + poly(A) signal
cggccgtgattctagatgcataccctgtggatgatcatcactttaaggtgatcctgcactatggcacactggtaatcgacggggttacgccgaacatgatcgactatttcggacggccgtatgaaggcatcgccgtgttcgacggcaaaaagatcactgtaacagggaccctgtggaacggcaacaaaattatcgacgagcgcctgatcaaccccgacggctccctgctgttccgagtaaccatcaacggagtgaccggctggcggctgtgcgaacgcattctggcgtaaggccgcgactctagagtcggggcggccggccgcttcgagcagacatgataagatacattgatgagtttggacaaaccacaactagaatgcagtgaaaaaaatgctttatttgtgaaatttgtgatgctattgctttatttgtaaccattataagctgcaataaacaagttaacaacaacaattgcattcattttatgtttcaggttcagggggaggtgtgggaggttttttaaagcaagtaaaacctctacaaatgtggtaaaatcgataaggatccgcgtatggtgcactc

SEQ ID NO: 54 - DNA, 866 bp, Artificial Sequence
  3'DTA + poly(A) signal
tgatagggataacagggtaatgcatcttttgtgatggaaaacttttcttcgtaccacgggactaaacctggttatgtagattccattcaaaaaggtatacaaaagccaaaatctggtacacaaggaaattatgacgatgattggaaagggttttatagtaccgacaataaatacgacgctgcgggatactctgtagataatgaaaacccgctctctggaaaagctggaggcgtggtcaaagtgacgtatccaggactgacgaaggttctcgcactaaaagtggataatgccgaaactattaagaaagagttaggtttaagtctcactgaaccgttgatggagcaagtcggaacggaagagtttatcaaaaggttcggtgatggtgcttcgcgtgtagtgctcagccttcccttcgctgaggggagttctagcgttgaatatattaataactgggaacaggcgaaagcgttaagcgtagaacttgagattaattttgaaacccgtggaaaacgtggccaagatgcgatgtatgagtatatggctcaagcctgtgcaggaaatcgtgtcaggcgatctttgtgattctagagtcggggcggccggccgcttcgagcagacatgataagatacattgatgagtttggacaaaccacaactagaatgcagtgaaaaaaatgctttatttgtgaaatttgtgatgctattgctttatttgtaaccattataagctgcaataaacaagttaacaacaacaattgcattcattttatgtttcaggttcagggggaggtgtgggaggttttttaaagcaagtaaaacctctacaaatgtggtaaaatcgataaggatccgcgtatggtgcactc

SEQ ID NO: 55 - DNA, 1131 bp, herpes simplex virus
  CDS (1)..(1131)
atggcttcgtaccccggccatcaacacgcgtctgcgttcgaccaggctgcgcgttctcgcggccatagcaaccgacgtacggcgttgcgccctcgccggcagcaagaagccacggaagtccgcccggagcagaaaatgcccacgctactgcgggtttatatagacggtccccacgggatggggaaaaccaccaccacgcaactgctggtggccctgggttcgcgcgacgatatcgtctacgtacccgagccgatgacttactggcgggtgctgggggcttccgagacaatcgcgaacatctacaccacacaacaccgcctcgaccagggtgagatatcggccggggacgcggcggtggtaatgacaagcgcccagataacaatgggcatgccttatgccgtgaccgacgccgttctggctcctcatatcgggggggaggctgggagctcacatgccccgcccccggccctcaccctcatcttcgaccgccatcccatcgccgccctcctgtgctacccggccgcgcggtaccttatgggcagcatgaccccccaggccgtgctggcgttcgtggccctcatcccgccgaccttgcccggcaccaacatcgtgcttggggcccttccggaggacagacacatcgaccgcctggccaaacgccagcgccccggcgagcggctggacctggctatgctggctgcgattcgccgcgtttacgggctacttgccaatacggtgcggtatctgcagtgcggcgggtcgtggcgggaggactggggacagctttcggggacggccgtgccgccccagggtgccgagccccagagcaacgcgggcccacgaccccatatcggggacacgttatttaccctgtttcgggcccccgagttgctggcccccaacggcgacctgtataacgtgtttgcctgggccttggacgtcttggccaaacgcctccgttccatgcacgtctttatcctggattacgaccaatcgcccgccggctgccgggacgccctgctgcaacttacctccgggatggtccagacccacgtcaccacccccggctccataccgacgatatgcgacctggcgcgcacgtttgcccgggagatgggggaggctaactga

SEQ ID NO: 56 - protein, 376 aa, herpes simplex virus
MASYPGHQHASAFDQAARSRGHSNRRTALRPRRQQEATEVRPEQKMPTLLRVYIDGPHGMGKTTTTQLLVALGSRDDIVYVPEPMTYWRVLGASETIANIYTTQHRLDQGEISAGDAAVVMTSAQITMGMPYAVTDAVLAPHIGGEAGSSHAPPPALTLIFDRHPIAALLCYPAARYLMGSMTPQAVLAFVALIPPTLPGTNIVLGALPEDRHIDRLAKRQRPGERLDLAMLAAIRRVYGLLANTVRYLQCGGSWREDWGQLSGTAVPPQGAEPQSNAGPRPHIGDTLFTLFRAPELLAPNGDLYNVFAWALDVLAKRLRSMHVFILDYDQSPAGCRDALLQLTSGMVQTHVTTPGSIPTICDLARTFAREMGEAN

SEQ ID NO: 57 - DNA, 129 bp, Artificial Sequence
  5'TK fragment
  CDS (1)..(129)
atggcttcgtaccccggccatcaacacgcgtctgcgttcgaccaggctgcgcgttctcgcggccatagcaaccgacgtacggcgttgcgccctcgccggcagcaagaagccacggaagtccgcctctga

SEQ ID NO: 58 - protein, 42 aa, Artificial Sequence
  Synthetic Construct
MASYPGHQHASAFDQAARSRGHSNRRTALRPRRQQEATEVRL

SEQ ID NO: 59 - DNA, 1107 bp, Artificial Sequence
  3'TK fragment
  CDS (1)..(1107)
cacgcgtctgcgttcgaccaggctgcgcgttctcgcggccatagcaaccgacgtacggcgttgcgccctcgccggcagcaagaagccacggaagtccgcccggagcagaaaatgcccacgctactgcgggtttatatagacggtccccacgggatggggaaaaccaccaccacgcaactgctggtggccctgggttcgcgcgacgatatcgtctacgtacccgagccgatgacttactggcgggtgctgggggcttccgagacaatcgcgaacatctacaccacacaacaccgcctcgaccagggtgagatatcggccggggacgcggcggtggtaatgacaagcgcccagataacaatgggcatgccttatgccgtgaccgacgccgttctggctcctcatatcgggggggaggctgggagctcacatgccccgcccccggccctcaccctcatcttcgaccgccatcccatcgccgccctcctgtgctacccggccgcgcggtaccttatgggcagcatgaccccccaggccgtgctggcgttcgtggccctcatcccgccgaccttgcccggcaccaacatcgtgcttggggcccttccggaggacagacacatcgaccgcctggccaaacgccagcgccccggcgagcggctggacctggctatgctggctgcgattcgccgcgtttacgggctacttgccaatacggtgcggtatctgcagtgcggcgggtcgtggcgggaggactggggacagctttcggggacggccgtgccgccccagggtgccgagccccagagcaacgcgggcccacgaccccatatcggggacacgttatttaccctgtttcgggcccccgagttgctggcccccaacggcgacctgtataacgtgtttgcctgggccttggacgtcttggccaaacgcctccgttccatgcacgtctttatcctggattacgaccaatcgcccgccggctgccgggacgccctgctgcaacttacctccgggatggtccagacccacgtcaccacccccggctccataccgacgatatgcgacctggcgcgcacgtttgcccgggagatgggggaggctaactga

SEQ ID NO: 60 - protein, 368 aa, Artificial Sequence
  Synthetic Construct
HASAFDQAARSRGHSNRRTALRPRRQQEATEVRPEQKMPTLLRVYIDGPHGMGKTTTTQLLVALGSRDDIVYVPEPMTYWRVLGASETIANIYTTQHRLDQGEISAGDAAVVMTSAQITMGMPYAVTDAVLAPHIGGEAGSSHAPPPALTLIFDRHPIAALLCYPAARYLMGSMTPQAVLAFVALIPPTLPGTNIVLGALPEDRHIDRLAKRQRPGERLDLAMLAAIRRVYGLLANTVRYLQCGGSWREDWGQLSGTAVPPQGAEPQSNAGPRPHIGDTLFTLFRAPELLAPNGDLYNVFAWALDVLAKRLRSMHVFILDYDQSPAGCRDALLQLTSGMVQTHVTTPGSIPTICDLARTFAREMGEAN

SEQ ID NO: 61 - DNA, 33 bp, Artificial Sequence
  sequence between 5'TK fragment and 3'TK fragment
tgattctcgagtagggataacagggtaatgcat

SEQ ID NO: 62 - DNA, 600 bp, Artificial Sequence
  SecNluc gene
  CDS (1)..(600)
atgaactccttctccacaagcgccttcggtccagttgccttctccctgggcctgctcctggtgttgcctgctgccttccctgccccagtcttcacactcgaagatttcgttggggactggcgacagacagccggctacaacctggaccaagtccttgaacagggaggtgtgtccagtttgtttcagaatctcggggtgtccgtaactccgatccaaaggattgtcctgagcggtgaaaatgggctgaagatcgacatccatgtcatcatcccgtatgaaggtctgagcggcgaccaaatgggccagatcgaaaaaatttttaaggtggtgtaccctgtggatgatcatcactttaaggtgatcctgcactatggcacactggtaatcgacggggttacgccgaacatgatcgactatttcggacggccgtatgaaggcatcgccgtgttcgacggcaaaaagatcactgtaacagggaccctgtggaacggcaacaaaattatcgacgagcgcctgatcaaccccgacggctccctgctgttccgagtaaccatcaacggagtgaccggctggcggctgtgcgaacgcattctggcgtaa

SEQ ID NO: 63 - protein, 199 aa, Artificial Sequence
  Synthetic Construct
MNSFSTSAFGPVAFSLGLLLVLPAAFPAPVFTLEDFVGDWRQTAGYNLDQVLEQGGVSSLFQNLGVSVTPIQRIVLSGENGLKIDIHVIIPYEGLSGDQMGQIEKIFKVVYPVDDHHFKVILHYGTLVIDGVTPNMIDYFGRPYEGIAVFDGKKITVTGTLWNGNKIIDERLINPDGSLLFRVTINGVTGWRLCERILA

SEQ ID NO: 64 - DNA, 432 bp, Artificial Sequence
  5'SecNluc fragment
  CDS (1)..(432)
atgaactccttctccacaagcgccttcggtccagttgccttctccctgggcctgctcctggtgttgcctgctgccttccctgccccagtcttcacactcgaagatttcgttggggactggcgacagacagccggctacaacctggaccaagtccttgaacagggaggtgtgtccagtttgtttcagaatctcggggtgtccgtaactccgatccaaaggattgtcctgagcggtgaaaatgggctgaagatcgacatccatgtcatcatcccgtatgaaggtctgagcggcgaccaaatgggccagatcgaaaaaatttttaaggtggtgtaccctgtggatgatcatcactttaaggtgatcctgcactatggcacactggtaatcgacggggttacgccgaacatgatcgactatttcggacggccgtga

SEQ ID NO: 65 - protein, 143 aa, Artificial Sequence
  Synthetic Construct
MNSFSTSAFGPVAFSLGLLLVLPAAFPAPVFTLEDFVGDWRQTAGYNLDQVLEQGGVSSLFQNLGVSVTPIQRIVLSGENGLKIDIHVIIPYEGLSGDQMGQIEKIFKVVYPVDDHHFKVILHYGTLVIDGVTPNMIDYFGRP

SEQ ID NO: 66 - DNA, 63 bp, Artificial Sequence
  primer TK-Fw
taatacgactcactataggctagcctcgagatccaccggtcatggcttcgtaccccggccatc

SEQ ID NO: 67 - DNA, 45 bp, Artificial Sequence
  primer TK-Rv
ccgccccgactctagagtcgcggtcagttagcctcccccatctcc

SEQ ID NO: 68 - DNA, 50 bp, Artificial Sequence
  primer SA-5'Nluc-40-Rv
atgcattaccctgttatccctatcatattacggacaccccgagattctga

SEQ ID NO: 69 - DNA, 49 bp, Artificial Sequence
  primer SA-3'Nluc-40-Fw
gggataacagggtaatgcatcggtgtgtccagtttgtttcagaatctcg

SEQ ID NO: 70 - DNA, 62 bp, Artificial Sequence
  primer SA-3'Nluc-40-90%-Fw
gggataacagggtaatgcatcggtgtgtctagtttgttccagaatctgggggtgtctgtaac

SEQ ID NO: 71 - DNA, 62 bp, Artificial Sequence
  primer SA-3'Nluc-40-70%-Fw
gggataacagggtaatgcatcggagtctctagcttattccaaaacctgggcgtctctgtaac

SEQ ID NO: 72 - DNA, 65 bp, Artificial Sequence
  primer SA-3'Nluc-40-60%-Fw
gggataacagggtaatgcatcggagtcagcagcttactccaaaacctgggcgtcagcgtgactcc

SEQ ID NO: 73 - DNA, 65 bp, Artificial Sequence
  primer SA-3'Nluc-40-50%-Fw
gggataacagggtaatgcatcggagtcagctctctcctccaaaacttggccgtcagcgtgactcc

SEQ ID NO: 74 - DNA, 126 bp, Artificial Sequence
  5'Nluc-40 fragment
  CDS (1)..(126)
atggtcttcacactcgaagatttcgttggggactggcgacagacagccggctacaacctggaccaagtccttgaacagggaggtgtgtccagtttgtttcagaatctcggggtgtccgtaatatga

SEQ ID NO: 75 - protein, 41 aa, Artificial Sequence
  Synthetic Construct
MVFTLEDFVGDWRQTAGYNLDQVLEQGGVSSLFQNLGVSVI

SEQ ID NO: 76 - protein, 144 aa, Artificial Sequence
  3'Nluc-40 protein encoded by 3'Nluc-40 fragment (homology 100%), 3'Nluc-40 fragment (homology 90%) and 3'Nluc-40 fragment (homology 70%)
GVSSLFQNLGVSVTPIQRIVLSGENGLKIDIHVIIPYEGLSGDQMGQIEKIFKVVYPVDDHHFKVILHYGTLVIDGVTPNMIDYFGRPYEGIAVFDGKKITVTGTLWNGNKIIDERLINPDGSLLFRVTINGVTGWRLCERILA

SEQ ID NO: 77 - protein, 144 aa, Artificial Sequence
  3'Nluc-40 protein encoded by 3'Nluc-40 fragment (homology 60%)
GVSSLLQNLGVSVTPIQRIVLSGENGLKIDIHVIIPYEGLSGDQMGQIEKIFKVVYPVDDHHFKVILHYGTLVIDGVTPNMIDYFGRPYEGIAVFDGKKITVTGTLWNGNKIIDERLINPDGSLLFRVTINGVTGWRLCERILA

SEQ ID NO: 78 - protein, 144 aa, Artificial Sequence
  3'Nluc-40 protein encoded by 3'Nluc-40 fragment (homology 50%)
GVSSLLQNLAVSVTPIQRIVLSGENGLKIDIHVIIPYEGLSGDQMGQIEKIFKVVYPVDDHHFKVILHYGTLVIDGVTPNMIDYFGRPYEGIAVFDGKKITVTGTLWNGNKIIDERLINPDGSLLFRVTINGVTGWRLCERILA

SEQ ID NO: 79 - DNA, 435 bp, Artificial Sequence
  3'Nluc-40 fragment (homology 100%)
ggtgtgtccagtttgtttcagaatctcggggtgtccgtaactccgatccaaaggattgtcctgagcggtgaaaatgggctgaagatcgacatccatgtcatcatcccgtatgaaggtctgagcggcgaccaaatgggccagatcgaaaaaatttttaaggtggtgtaccctgtggatgatcatcactttaaggtgatcctgcactatggcacactggtaatcgacggggttacgccgaacatgatcgactatttcggacggccgtatgaaggcatcgccgtgttcgacggcaaaaagatcactgtaacagggaccctgtggaacggcaacaaaattatcgacgagcgcctgatcaaccccgacggctccctgctgttccgagtaaccatcaacggagtgaccggctggcggctgtgcgaacgcattctggcgtaa

SEQ ID NO: 80 - DNA, 435 bp, Artificial Sequence
  3'Nluc-40 fragment (homology 90%)
ggtgtgtctagtttgttccagaatctgggggtgtctgtaactccgatccaaaggattgtcctgagcggtgaaaatgggctgaagatcgacatccatgtcatcatcccgtatgaaggtctgagcggcgaccaaatgggccagatcgaaaaaatttttaaggtggtgtaccctgtggatgatcatcactttaaggtgatcctgcactatggcacactggtaatcgacggggttacgccgaacatgatcgactatttcggacggccgtatgaaggcatcgccgtgttcgacggcaaaaagatcactgtaacagggaccctgtggaacggcaacaaaattatcgacgagcgcctgatcaaccccgacggctccctgctgttccgagtaaccatcaacggagtgaccggctggcggctgtgcgaacgcattctggcgtaa

SEQ ID NO: 81 - DNA, 435 bp, Artificial Sequence
  3'Nluc-40 fragment (homology 70%)
ggagtctctagcttattccaaaacctgggcgtctctgtaactccgatccaaaggattgtcctgagcggtgaaaatgggctgaagatcgacatccatgtcatcatcccgtatgaaggtctgagcggcgaccaaatgggccagatcgaaaaaatttttaaggtggtgtaccctgtggatgatcatcactttaaggtgatcctgcactatggcacactggtaatcgacggggttacgccgaacatgatcgactatttcggacggccgtatgaaggcatcgccgtgttcgacggcaaaaagatcactgtaacagggaccctgtggaacggcaacaaaattatcgacgagcgcctgatcaaccccgacggctccctgctgttccgagtaaccatcaacggagtgaccggctggcggctgtgcgaacgcattctggcgtaa

SEQ ID NO: 82 - DNA, 435 bp, Artificial Sequence
  3'Nluc-40 fragment (homology 60%)
ggagtcagcagcttactccaaaacctgggcgtcagcgtgactccgatccaaaggattgtcctgagcggtgaaaatgggctgaagatcgacatccatgtcatcatcccgtatgaaggtctgagcggcgaccaaatgggccagatcgaaaaaatttttaaggtggtgtaccctgtggatgatcatcactttaaggtgatcctgcactatggcacactggtaatcgacggggttacgccgaacatgatcgactatttcggacggccgtatgaaggcatcgccgtgttcgacggcaaaaagatcactgtaacagggaccctgtggaacggcaacaaaattatcgacgagcgcctgatcaaccccgacggctccctgctgttccgagtaaccatcaacggagtgaccggctggcggctgtgcgaacgcattctggcgtaa

SEQ ID NO: 83 - DNA, 435 bp, Artificial Sequence
  3'Nluc-40 fragment (homology 50%)
ggagtcagctctctcctccaaaacttggccgtcagcgtgactccgatccaaaggattgtcctgagcggtgaaaatgggctgaagatcgacatccatgtcatcatcccgtatgaaggtctgagcggcgaccaaatgggccagatcgaaaaaatttttaaggtggtgtaccctgtggatgatcatcactttaaggtgatcctgcactatggcacactggtaatcgacggggttacgccgaacatgatcgactatttcggacggccgtatgaaggcatcgccgtgttcgacggcaaaaagatcactgtaacagggaccctgtggaacggcaacaaaattatcgacgagcgcctgatcaaccccgacggctccctgctgttccgagtaaccatcaacggagtgaccggctggcggctgtgcgaacgcattctggcgtaa